European Patent Application EP 4 484 558 A1, published January 1, 2025. Title: 一种优化的Cas蛋白及其应用. Applicant: 山东舜丰生物科技有限公司. The sequence listing filed with the application follows.

SEQUENCE LISTING (4 sequences)

SEQ ID NO: 1 - protein, 1045 aa, synthetic construct
  REGION 1..1045: note = Cas12i
MKKVEVSRPYQSLLLPNHRKFKYLDETWNAYKSVKSLLHRFLVCAYGAVPFNKFVEVVEKVDNDQLVLAFAVRLFRLVPVESTSFAKVDKANLAKSLANHLPVGTAIPANVQSYFDSNFDPKKYMWIDCAWEADRLAREMGLSASQFSEYATTMLWEDWLPLNKDDVNGWGSVSGLFGEGKKEDRQQKVKMLNNLLNGIKKNPPKDYTQYLKILLNAFDAKSHKEAVKNYKGDSTGRTASYLSEKSGEITELMLEQLMSNIQRDIGDKQKEISLPKKDVVKKYLESESGVPYDQNLWSQAYRNAASSIKKTDTRNFNSTLEKFKNEVELRGLLSEGDDVEILRSKFFSSEFHKTPDKFVIKPEHIGFNNKYNVVAELYKLKAEATDFESAFATVKDEFEEKGIKHPIKNILEYIWNNEVPVEKWGRVARFNQSEEKLLRIKANPTVECNQGMTFGNSAMVGEVLRSNYVSKKGALVSGEHGGRLIGQNNMIWLEMRLLNKGKWETHHVPTHNMKFFEEVHAYNPSLADSVNVRNRLYRSEDYTQLPSSITDGLKGNPKAKLLKRQHCALNNMTANVLNPKLSFTINKKNDDYTVIIVHSVEVSKPRREVLVGDYLVGMDQNQTASNTYAVMQVVKPKSTDAIPFRNMWVRFVESGSIESRTLNSRGEYVDQLNHDGVDLFEIGDTEWVDSARKFFNKLGVKHKDGTLVDLSTAPRKAYAFNNFYFKTMLNHLRSNEVDLTLLRNEILRVANGRFSPMRLGSLSWTTLKALGSFKSLVLSYFDRLGAKEMVDKEAKDKSLFDLLVAINNKRSNKREERTSRIASSLMTVAQKYKVDNAVVHVVVEGNLSSTDRSASKAHNRNTMDWCSRAVVKKLEDMCNLYGFNIKGVPAFYTSHQDPLVHRADYDDPKPALRCRYSSYSRADFSKWGQNALAAVVRWASNKKSNTCYKVGAVEFLKQHGLFADKKLTVEQFLSKVKDEEILIPRRGGRVFLTTHRLLAESTFVYLNGVKYHSCNADEVAAVNICLNDWVIPCKKKMKEESSASG

SEQ ID NO: 2 - DNA, 3138 bp, synthetic construct
  misc_feature 1..3138: note = Cas12i
  source 1..3138: mol_type = other DNA
atgaagaaggtcgaggtgtcgcggccataccagagcctgctcctgccaaaccaccggaagttcaagtacctcgacgagacctggaatgcgtacaagtccgttaagagcctgctccaccgcttcctggtgtgcgcttacggcgctgttcccttcaacaagttcgtggaggttgtcgagaaggttgataacgaccagctcgtgctggctttcgcggtgcgcctcttccgcctggtccccgtggagagcacctctttcgccaaggttgacaaggccaatctggcgaagtccctggccaatcacctgcctgtgggcacagccattcctgccaatgttcagtcctacttcgattcaaatttcgaccccaagaagtacatgtggatcgactgcgcgtgggaggctgatcgcctggctcgggagatgggcctgagcgcgagccagttctctgagtacgcgactacaatgctctgggaggactggctgcccctcaataaggatgatgtgaacggctgggggtccgtgtcggggctcttcggcgagggcaagaaggaggaccggcagcagaaggtgaagatgctgaataacctgctgaatggcatcaagaagaatccgcccaaggattacacccagtacctgaagatcctcctgaacgcgttcgacgcgaagtcgcacaaggaggctgttaagaactacaagggggactctacggggcgcaccgcgtcttacctgtcagagaagtctggcgagatcacagagctgatgctcgagcagctgatgtcaaacatccagagggatattggcgacaagcagaaggagatctccctgccgaagaaggacgtggtcaagaagtacctcgagtcagagtccggcgtcccatacgatcagaacctgtggtcccaggcctaccgcaacgctgccagctcgatcaagaagactgatacgcggaacttcaactccactctcgagaagttcaagaatgaggtggagctgaggggcctgctgagcgagggcgacgacgttgagatcctgaggtctaagttcttcagcagcgagttccacaagacccctgataagttcgttattaagccagagcatattgggttcaacaataagtacaatgtcgttgccgagctgtacaagctcaaggctgaggcgaccgatttcgagagcgctttcgccacagtcaaggatgagttcgaggagaagggcatcaagcacccaatcaagaacatcctcgagtacatctggaataacgaggtgcccgtcgagaagtggggccgggttgcccgcttcaaccagtccgaggagaagctcctccggattaaggccaaccccacggtggagtgcaaccagggcatgaccttcggcaattccgcgatggttggcgaggtcctcaggtccaactacgtctctaagaagggcgcgctggtgtccggcgagcacggcgggcgcctgatcggccagaacaatatgatctggctggagatgcggctgctcaacaaggggaagtgggagacccaccacgttccaacccataacatgaagttcttcgaggaggtgcatgcctacaatccctctctggcggattctgttaacgtgcggaatcggctgtaccgctcagaggactacacccagctgccttcaagcattaccgacgggctgaagggcaatccgaaggcgaagctcctgaagcgccagcactgcgctctgaacaatatgacagctaatgttctcaatcctaagctgagcttcacgatcaacaagaagaacgatgattacacggtcatcattgtccatagcgttgaggtctcgaagcctcggagggaggtgctcgttggcgattacctcgtgggcatggaccagaatcagacagcgtctaatacatacgccgtcatgcaggtcgtcaagccgaagtctacagatgcgatcccgttccgcaacatgtgggtgcggttcgtggagtcagggtctatcgagtcccggaccctcaacagccgcggggagtatgttgatcagctgaatcatgacggcgtggacctcttcgagatcggcgatacggagtgggtggactccgcgcggaagttcttcaataagctcggcgttaagcacaaggatggcacactggttgatctgtctacggcgccccggaaggcctacgctttcaacaacttctacttcaagaccatgctgaatcatctccggagcaatgaggttgacctgacgctcctgcgcaatgagatcctccgggttgccaatgggcggttctccccgatgcgcctcggctcgctctcctggactactctcaaggccctgggctcgttcaagtccctggtgctgtcgtacttcgaccggctgggcgccaaggagatggtcgacaaggaggctaaggataagtctctcttcgacctcctcgtggctatcaacaacaagcgctctaataagcgcgaggagcggacttcccggattgcctccagcctcatgactgtggcgcagaagtacaaggttgataacgctgtggtccatgtggtcgtcgaggggaatctctccagcacggacaggagcgcgtcaaaggcccataatcggaacactatggattggtgctctagggccgtggtgaagaagctggaggacatgtgcaatctctacggcttcaatatcaagggcgtcccagccttctacacatcccaccaggacccgctcgtccaccgcgccgactacgatgaccctaagccggcgctcaggtgccgctactcctcgtactcaagggcggacttcagcaagtgggggcagaacgctctcgcggcggtggttcgctgggcgtctaataagaagtccaacacctgctacaaggtcggggccgtggagttcctcaagcagcacggcctcttcgcggacaagaagctgacagtcgagcagttcctctcgaaggtgaaggacgaggagatcctcattccccgcaggggcgggagggtgttcctcacaactcaccggctcctggcggagtccactttcgtgtacctgaacggcgttaagtaccattcatgcaacgccgatgaggtggcggctgttaacatctgcctgaatgactgggttatcccgtgcaagaagaagatgaaggaggagtcaagcgcgtccgggtaa

SEQ ID NO: 3 - protein, 1045 aa, synthetic construct
MKKVEVRRPYQSLLLPNHRKFKYLDETWNAYKSVKSLLHRFLVCAYGAVPFNKFVEVVEKVDNDQLVLAFAVRLFRLVPVESTSFAKVDKANLAKSLANHLPVGTAIPANVQSYFDSNFDPKKYMWIDCAWEADRLAREMGLSASQFSEYATTMLWEDWLPLNKDDVNGWGSVSGLFGEGKKEDRQQKVKMLNNLLNGIKKNPPKDYTQYLKILLNAFDAKSHKEAVKNYKGDSTGRTASYLSEKSGEITELMLEQLMSNIQRDIGDKQKEISLPKKDVVKKYLESESGVPYDQNLWSQAYRNAASSIKKTDTRNFNSTLEKFKNEVELRGLLSEGDDVEILRSKFFSSEFHKTPDKFVIKPEHIGFNNKYNVVAELYKLKAEATDFESAFATVKDEFEEKGIKHPIKNILEYIWNNEVPVEKWGRVARFNQSEEKLLRIKANPTVECNQGMTFGNSAMVGEVLRSNYVSKKGALVSGEHGGRLIGQNNMIWLEMRLLNKGKWETHHVPTHNMKFFEEVHAYNPSLADSVNVRNRLYRSEDYTQLPSSITDGLKGNPKAKLLKRQHCALNNMTANVLNPKLSFTINKKNDDYTVIIVHSVEVSKPRREVLVGDYLVGMDQNQTASNTYAVMQVVKPKSTDAIPFRNMWVRFVESGSIESRTLNSRGEYVDQLNHDGVDLFEIGDTEWVDSARKFFNKLGVKHKDGTLVDLSTAPRKAYAFNNFYFKTMLNHLRSNEVDLTLLRNEILRVANGRFSPMRLGSLSWTTLKALGSFKSLVLSYFDRLGAKEMVDKEAKDKSLFDLLVAINNKRSNKREERTSRIASSLMTVAQKYKVDNAVVHVVVEGNLSSTDRSASKAHNRNTMDWCSRAVVKKLEDMCNLYGFNIKGVPAFYTSHQDPLVHRADYDDPKPALRCRYSSYSRADFSKWGQNALAAVVRWASNKKSNTCYKVGAVEFLKQHGLFADKKLTVEQFLSKVKDEEILIPRRGGRVFLTTHRLLAESTFVYLNGVKYHSCNADEVAAVNICLNDWVIPCKKKMKEESSASG

SEQ ID NO: 4 - DNA, 3135 bp, synthetic construct
  source 1..3135: mol_type = other DNA
atgaagaaggtcgaggtgaggcggccataccagagcctgctcctgccaaaccaccggaagttcaagtacctcgacgagacgtggaatgcgtacaagtccgttaagagcctgctccaccgcttcctggtgtgcgcttacggcgctgttcccttcaacaagttcgtggaggttgtcgagaaggttgataacgaccagctcgtgctggctttcgcggtgcgcctcttccgcctggtccccgtggagagcacctctttcgccaaggttgacaaggccaatctggcgaagtccctggccaatcacctgcctgtgggcacagccattcctgccaatgttcagtcctacttcgattcaaatttcgaccccaagaagtacatgtggatcgactgcgcgtgggaggctgatcgcctggctcgggagatgggcctgagcgcgagccagttctctgagtacgcgactacaatgctctgggaggactggctgcccctcaataaggatgatgtgaacggctgggggtccgtgtcggggctcttcggcgagggcaagaaggaggaccggcagcagaaggtgaagatgctgaataacctgctgaatggcatcaagaagaatccgcccaaggattacacccagtacctgaagatcctcctgaacgcgttcgacgcgaagtcgcacaaggaggctgttaagaactacaagggggactctacggggcgcaccgcgtcttacctgtcagagaagtctggcgagatcacagagctgatgctcgagcagctgatgtcaaacatccagagggatatcggcgacaagcagaaggagatctccctgccgaagaaggacgtggtcaagaagtacctggagtcagagtccggcgtcccatacgatcagaacctgtggtcccaggcctaccgcaacgctgccagctcgatcaagaaaactgatacgcggaacttcaactccactctggagaagttcaagaatgaggtggagctgaggggcctcctgagcgagggcgacgacgttgagatcctgaggtctaagttcttcagcagcgagttccacaagacccctgataagttcgttattaagccagagcatattgggttcaacaataagtacaatgtcgttgccgagctgtacaagctcaaggctgaagcgaccgatttcgagagtgctttcgccacagtcaaggatgagttcgaggagaagggcatcaagcacccaatcaagaacatcctggagtacatctggaataacgaggtgcccgtcgagaagtggggccgggttgcccgcttcaaccagtccgaggagaagctcctccggattaaggccaaccccacggtggagtgcaaccagggcatgaccttcggcaattccgcgatggttggcgaggtcctcaggtccaactacgtctctaagaagggcgcgctggtgtccggcgagcacggcgggcgcctgatcggccagaacaatatgatctggctggagatgcggctgctcaacaaggggaagtgggagacgcaccacgttccaacccataacatgaagttcttcgaggaggtgcatgcctacaatccctctctggcggattctgttaacgtgcggaatcggctgtaccgctcagaggactacacccagctgccttcaagcattaccgacgggctgaagggcaatccgaaggcgaagctcctgaagcgccagcactgcgctctgaacaatatgacagctaatgttctcaatcctaagctgagcttcacgatcaacaagaagaacgatgattacacggtcatcattgtccatagcgttgaggtgtcgaagcctcggagggaggtgctcgttggcgattacctcgtgggcatggaccagaatcagacagcgtctaatacatacgccgtcatgcaggtcgtcaagccgaagtctacagatgcgatcccgttccgcaacatgtgggtgcggttcgtggagtcagggtctatcgagtcccggaccctcaacagccgcggggagtatgttgatcagctgaatcatgacggcgtggacctcttcgagatcggcgatacggagtgggtggactccgcgcggaagttcttcaataagctcggcgttaagcacaaggatggcacactggttgatctgtctacggcgccccggaaggcctacgctttcaacaacttctacttcaagaccatgctgaatcatctccggagcaatgaggttgacctgacgctcctgcgcaatgagatcctccgggttgccaatgggcggttctccccgatgcgcctcggctcgctctcctggactactctcaaggccctgggctcgttcaagtccctggtgctgtcgtacttcgaccggctgggcgccaaggagatggtcgacaaggaggctaaggataagtctctcttcgacctcctcgtggctatcaacaacaagcgctctaataagcgcgaggagcggacttcccggattgcctccagcctcatgactgtggcgcagaagtacaaggttgataacgctgtggtccatgtggtcgtcgaggggaatctctccagcacggacaggagcgcgtcaaaggcccataatcggaacactatggattggtgctctagggccgtggtgaagaagctggaggacatgtgcaatctctacggcttcaatatcaagggcgtcccagccttctacacatcccaccaggacccgctcgtccaccgcgccgactacgatgaccctaagccggcgctcaggtgccgctactcctcgtactcaagggcggacttcagcaagtgggggcagaacgctctcgcggcggtggttcgctgggcgtctaataagaagtccaacacctgctacaaggtcggggccgtggagttcctcaagcagcacggcctcttcgcggacaagaagctgacagtcgagcagttcctctcgaaggtgaaggacgaggagatcctcattccccgcaggggcgggagggtgttcctcacaactcaccggctcctggcggagtccactttcgtgtacctgaacggcgttaagtaccattcatgcaacgccgatgaggtggcggctgttaacatctgcctgaatgactgggttatcccgtgcaagaagaagatgaaggaggagtcaagcgcgtccggg